European Patent Specification EP 4 114 985 B1, published May 7, 2025. Title: COMPOSITIONS AND METHODS FOR DETECTING SARS-COV-2 NUCLEIC ACID. Applicant: Gen-Probe Incorporated. The sequence listing filed with the application follows.

SEQUENCE LISTING (115 sequences)

SEQ ID NO: 1 - DNA, 29882 bp, Coronavirus
  ref <308>: MT106054
  ref <309>: 2020-02-24
  ref <313>: (1)..(29882)
attaaaggtttataccttcccaggtaacaaaccaaccaactttcgatctcttgtagatctgttctctaaacgaactttaaaatctgtgtggctgtcactcggctgcatgcttagtgcactcacgcagtataattaataactaattactgtcgttgacaggacacgagtaactcgtctatcttctgcaggctgcttacggtttcgtccgtgttgcagccgatcatcagcacatctaggtttcgtccgggtgtgaccgaaaggtaagatggagagccttgtccctggtttcaacgagaaaacacacgtccaactcagtttgcctgttttacaggttcgcgacgtgctcgtacgtggctttggagactccgtggaggaggtcttatcagaggcacgtcaacatcttaaagatggcacttgtggcttagtagaagttgaaaaaggcgttttgcctcaacttgaacagccctatgtgttcatcaaacgttcggatgctcgaactgcacctcatggtcatgttatggttgagctggtagcagaactcgaaggcattcagtacggtcgtagtggtgagacacttggtgtccttgtccctcatgtgggcgaaataccagtggcttaccgcaaggttcttcttcgtaagaacggtaataaaggagctggtggccatagttacggcgccgatctaaagtcatttgacttaggcgacgagcttggcactgatccttatgaagattttcaagaaaactggaacactaaacatagcagtggtgttacccgtgaactcatgcgtgagcttaacggaggggcatacactcgctatgtcgataacaacttctgtggccctgatggctaccctcttgagtgcattaaagaccttctagcacgtgctggtaaagcttcatgcactttgtccgaacaactggactttattgacactaagaggggtgtatactgctgccgtgaacatgagcatgaaattgcttggtacacggaacgttctgaaaagagctatgaattgcagacaccttttgaaattaaattggcaaagaaatttgacaccttcaatggggaatgtccaaattttgtatttcccttaaattccataatcaagactattcaaccaagggttgaaaagaaaaagcttgatggctttatgggtagaattcgatctgtctatccagttgcgtcaccaaatgaatgcaaccaaatgtgcctttcaactctcatgaagtgtgatcattgtggtgaaacttcatggcagacgggcgattttgttaaagccacttgcgaattttgtggcactgagaatttgactaaagaaggtgccactacttgtggttacttaccccaaaatgctgttgttaaaatttattgtccagcatgtcacaattcagaagtaggacctgagcatagtcttgccgaataccataatgaatctggcttgaaaaccattcttcgtaagggtggtcgcactattgcctttggaggctgtgtgttctcttatgttggttgccataacaagtgtgcctattgggttccacgtgctagcgctaacataggttgtaaccatacaggtgttgttggagaaggttccgaaggtcttaatgacaaccttcttgaaatactccaaaaagagaaagtcaacatcaatattgttggtgactttaaacttaatgaagagatcgccattattttggcatctttttctgcttccacaagtgcttttgtggaaactgtgaaaggtttggattataaagcattcaaacaaattgttgaatcctgtggtaattttaaagttacaaaaggaaaagctaaaaaaggtgcctggaatattggtgaacagaaatcaatactgagtcctctttatgcatttgcatcagaggctgctcgtgttgtacgatcaattttctcccgcactcttgaaactgctcaaaattctgtgcgtgttttacagaaggccgctataacaatactagatggaatttcacagtattcactgagactcattgatgctatgatgttcacatctgatttggctactaacaatctagttgtaatggcctacattacaggtggtgttgttcagttgacttcgcagtggctaactaacatctttggcactgtttatgaaaaactcaaacccgtccttgattggcttgaagagaagtttaaggaaggtgtagagtttcttagagacggttgggaaattgttaaatttatctcaacctgtgcttgtgaaattgtcggtggacaaattgtcacctgtgcaaaggaaattaaggagagtgttcagacattctttaagcttgtaaataaatttttggctttgtgtgctgactctatcattattggtggagctaaacttaaagccttgaatttaggtgaaacatttgtcacgcactcaaagggattgtacagaaagtgtgttaaatccagagaagaaactggcctactcatgcctctaaaagccccaaaagaaattatcttcttagagggagaaacacttcccacagaagtgttaacagaggaagttgtcttgaaaactggtgatttacaaccattagaacaacctactagtgaagctgttgaagctccattggttggtacaccagtttgtattaacgggcttatgttgctcgaaatcaaagacacagaaaagtactgtgcccttgcacctaatatgatggtaacaaacaataccttcacactcaaaggcggtgcaccaacaaaggttacttttggtgatgacactgtgatagaagtgcaaggttacaagagtgtgaatatcacttttgaacttgatgaaaggattgataaagtacttaatgagaagtgctctgcctatacagttgaactcggtacagaagtaaatgagttcgcctgtgttgtggcagatgctgtcataaaaactttgcaaccagtatctgaattacttacaccactgggcattgatttagatgagtggagtatggctacatactacttatttgatgagtctggtgagtttaaattggcttcacatatgtattgttctttctaccctccagatgaggatgaagaagaaggtgattgtgaagaagaagagtttgagccatcaactcaatatgagtatggtactgaagatgattaccaaggtaaacctttggaatttggtgccacttctgctgctcttcaacctgaagaagagcaagaagaagattggttagatgatgatagtcaacaaactgttggtcaacaagacggcagtgaggacaatcagacaactactattcaaacaattgttgaggttcaacctcaattagagatggaacttacaccagttgttcagactattgaagtgaatagttttagtggttatttaaaacttactgacaatgtatacattaaaaatgcagacattgtggaagaagctaaaaaggtaaaaccaacagtggttgttaatgcagccaatgtttaccttaaacatggaggaggtgttgcaggagccttaaataaggctactaacaatgccatgcaagttgaatctgatgattacatagctactaatggaccacttaaagtgggtggtagttgtgttttaagcggacacaatcttgctaaacactgtcttcatgttgtcggcccaaatgttaacaaaggtgaagacattcaacttcttaagagtgcttatgaaaattttaatcagcacgaagttctacttgcaccattattatcagctggtatttttggtgctgaccctatacattctttaagagtttgtgtagatactgttcgcacaaatgtctacttagctgtctttgataaaaatctctatgacaaacttgtttcaagctttttggaaatgaagagtgaaaagcaagttgaacaaaagatcgctgagattcctaaagaggaagttaagccatttataactgaaagtaaaccttcagttgaacagagaaaacaagatgataagaaaatcaaagcttgtgttgaagaagttacaacaactctggaagaaactaagttcctcacagaaaacttgttactttatattgacattaatggcaatcttcatccagattctgccactcttgttagtgacattgacatcactttcttaaagaaagatgctccatatatagtgggtgatgttgttcaagagggtgttttaactgctgtggttatacctactaaaaaggctggtggcactactgaaatgctagcgaaagctttgagaaaagtgccaacagacaattatataaccacttacccgggtcagggtttaaatggttacactgtagaggaggcaaagacagtgcttaaaaagtgtaaaagtgccttttacattctaccatctattatctctaatgagaagcaagaaattcttggaactgtttcttggaatttgcgagaaatgcttgcacatgcagaagaaacacgcaaattaatgcctgtctgtgtggaaactaaagccatagtttcaactatacagcgtaaatataagggtattaaaatacaagagggtgtggttgattatggtgctagattttacttttacaccagtaaaacaactgtagcgtcacttatcaacacacttaacgatctaaatgaaactcttgttacaatgccacttggctatgtaacacatggcttaaatttggaagaagctgctcggtatatgagatctctcaaagtgccagctacagtttctgtttcttcacctgatgctgttacagcgtataatggttatcttacttcttcttctaaaacacctgaagaacattttattgaaaccatctcacttgctggttcctataaagattggtcctattctggacaatctacacaactaggtatagaatttcttaagagaggtgataaaagtgtatattacactagtaatcctaccacattccacctagatggtgaagttatcacctttgacaatcttaagacacttctttctttgagagaagtgaggactattaaggtgtttacaacagtagacaacattaacctccacacgcaagttgtggacatgtcaatgacatatggacaacagtttggtccaacttatttggatggagctgatgttactaaaataaaacctcataattcacatgaaggtaaaacattttatgttttacctaatgatgacactctacgtgttgaggcttttgagtactaccacacaactgatcctagttttctgggtaggtacatgtcagcattaaatcacactaaaaagtggaaatacccacaagttaatggtttaacttctattaaatgggcagataacaactgttatcttgccactgcattgttaacactccaacaaatagagttgaagtttaatccacctgctctacaagatgcttattacagagcaagggctggtgaagctgctaacttttgtgcacttatcttagcctactgtaataagacagtaggtgagttaggtgatgttagagaaacaatgagttacttgtttcaacatgccaatttagattcttgcaaaagagtcttgaacgtggtgtgtaaaacttgtggacaacagcagacaacccttaagggtgtagaagctgttatgtacatgggcacactttcttatgaacaatttaagaaaggtgttcagataccttgtacgtgtggtaaacaagctacaaaatatctagtacaacaggagtcaccttttgttatgatgtcagcaccacctgctcagtatgaacttaagcatggtacatttacttgtgctagtgagtacactggtaattaccagtgtggtcactataaacatataacttctaaagaaactttgtattgcatagacggtgctttacttacaaagtcctcagaatacaaaggtcctattacggatgttttctacaaagaaaacagttacacaacaaccataaaaccagttacttataaattggatggtgttgtttgtacagaaattgaccctaagttggacaattattataagaaagacaattcttatttcacagagcaaccaattgatcttgtaccaaaccaaccatatccaaacgcaagcttcgataattttaagtttgtatgtgataatatcaaatttgctgatgatttaaaccagttaactggttataagaaacctgcttcaagagagcttaaagttacatttttccctgacttaaatggtgatgtggtggctattgattataaacactacacaccctcttttaagaaaggagctaaattgttacataaacctattgtttggcatgttaacaatgcaactaataaagccacgtataaaccaaatacctggtgtatacgttgtctttggagcacaaaaccagttgaaacatcaaattcgtttgatgtactgaagtcagaggacgcgcagggaatggataatcttgcctgcgaagatctaaaaccagtctctgaagaagtagtggaaaatcctaccatacagaaagacgttcttgagtgtaatgtgaaaactaccgaagttgtaggagacattatacttaaaccagcaaataatagtttaaaaattacagaagaggttggccacacagatctaatggctgcttatgtagacaattctagtcttactattaagaaacctaatgaattatctagagtattaggtttgaaaacccttgctactcatggtttagctgctgttaatagtgtcccttgggatactatagctaattatgctaagccttttcttaacaaagttgttagtacaactactaacatagttacacggtgtttaaaccgtgtttgtactaattatatgccttatttctttactttattgctacaattgtgtacttttactagaagtacaaattctagaattaaagcatctatgccgactactatagcaaagaatactgttaagagtgtcggtaaattttgtctagaggcttcatttaattatttgaagtcacctaatttttctaaactgataaatattataatttggtttttactattaagtgtttgcctaggttctttaatctactcaaccgctgctttaggtgttttaatgtctaatttaggcatgccttcttactgtactggttacagagaaggctatttgaactctactaatgtcactattgcaacctactgtactggttctataccttgtagtgtttgtcttagtggtttagattctttagacacctatccttctttagaaactatacaaattaccatttcatcttttaaatgggatttaactgcttttggcttagttgcagagtggtttttggcatatattcttttcactaggtttttctatgtacttggattggctgcaatcatgcaattgtttttcagctattttgcagtacattttattagtaattcttggcttatgtggttaataattaatcttgtacaaatggccccgatttcagctatggttagaatgtacatcttctttgcatcattttattatgtatggaaaagttatgtgcatgttgtagacggttgtaattcatcaacttgtatgatgtgttacaaacgtaatagagcaacaagagtcgaatgtacaactattgttaatggtgttagaaggtccttttatgtctatgctaatggaggtaaaggcttttgcaaactacacaattggaattgtgttaattgtgatacattctgtgctggtagtacatttattagtgatgaagttgcgagagacttgtcactacagtttaaaagaccaataaatcctactgaccagtcttcttacatcgttgatagtgttacagtgaagaatggttccatccatctttactttgataaagctggtcaaaagacttatgaaagacattctctctctcattttgttaacttagacaacctgagagctaataacactaaaggttcattgcctattaatgttatagtttttgatggtaaatcaaaatgtgaagaatcatctgcaaaatcagcgtctgtttactacagtcagcttatgtgtcaacctatactgttactagatcaggcattagtgtctgatgttggtgatagtgcggaagttgcagttaaaatgtttgatgcttacgttaatacgttttcatcaacttttaacgtaccaatggaaaaactcaaaacactagttgcaactgcagaagctgaacttgcaaagaatgtgtccttagacaatgtcttatctacttttatttcagcagctcggcaagggtttgttgattcagatgtagaaactaaagatgttgttgaatgtcttaaattgtcacatcaatctgacatagaagttactggcgatagttgtaataactatatgctcacctataacaaagttgaaaacatgacaccccgtgaccttggtgcttgtattgactgtagtgcgcgtcatattaatgcgcaggtagcaaaaagtcacaacattgctttgatatggaacgttaaagatttcatgtcattgtctgaacaactacgaaaacaaatacgtagtgctgctaaaaagaataacttaccttttaagttgacatgtgcaactactagacaagttgttaatgttgtaacaacaaagatagcacttaagggtggtaaaattgttaataattggttgaagcagttaattaaagttacacttgtgttcctttttgttgctgctattttctatttaataacacctgttcatgtcatgtctaaacatactgacttttcaagtgaaatcataggatacaaggctattgatggtggtgtcactcgtgacatagcatctacagatacttgttttgctaacaaacatgctgattttgacacatggtttagtcagcgtggtggtagttatactaatgacaaagcttgcccattgattgctgcagtcataacaagagaagtgggttttgtcgtgcctggtttgcctggcacgatattacgcacaactaatggtgactttttgcatttcttacctagagtttttagtgcagttggtaacatctgttacacaccatcaaaacttatagagtacactgactttgcaacatcagcttgtgttttggctgctgaatgtacaatttttaaagatgcttctggtaagccagtaccatattgttatgataccaatgtactagaaggttctgttgcttatgaaagtttacgccctgacacacgttatgtgctcatggatggctctattattcaatttcctaacacctaccttgaaggttctgttagagtggtaacaacttttgattctgagtactgtaggcacggcacttgtgaaagatcagaagctggtgtttgtgtatctactagtggtagatgggtacttaacaatgattattacagatctttaccaggagttttctgtggtgtagatgctgtaaatttacttactaatatgtttacaccactaattcaacctattggtgctttggacatatcagcatctatagtagctggtggtattgtagctatcgtagtaacatgccttgcctactattttatgaggtttagaagagcttttggtgaatacagtcatgtagttgcctttaatactttactattccttatgtcattcactgtactctgtttaacaccagtttactcattcttacctggtgtttattctgttatttacttgtacttgacattttatcttactaatgatgtttcttttttagcacatattcagtggatggttatgttcacacctttagtacctttctggataacaattgcttatatcatttgtatttccacaaagcatttctattggttctttagtaattacctaaagagacgtgtagtctttaatggtgtttcctttagtacttttgaagaagctgcgctgtgcacctttttgttaaataaagaaatgtatctaaagttgcgtagtgatgtgctattacctcttacgcaatataatagatacttagctctttataataagtacaagtattttagtggagcaatggatacaactagctacagagaagctgcttgttgtcatctcgcaaaggctctcaatgacttcagtaactcaggttctgatgttctttaccaaccaccacaaacctctatcacctcagctgttttgcagagtggttttagaaaaatggcattcccatctggtaaagttgagggttgtatggtacaagtaacttgtggtacaactacacttaacggtctttggcttgatgacgtagtttactgtccaagacatgtgatctgcacctctgaagacatgcttaaccctaattatgaagatttactcattcgtaagtctaatcataatttcttggtacaggctggtaatgttcaactcagggttattggacattctatgcaaaattgtgtacttaagcttaaggttgatacagccaatcctaagacacctaagtataagtttgttcgcattcaaccaggacagactttttcagtgttagcttgttacaatggttcaccatctggtgtttaccaatgtgctatgaggcccaatttcactattaagggttcattccttaatggttcatgtggtagtgttggttttaacatagattatgactgtgtctctttttgttacatgcaccatatggaattaccaactggagttcatgctggcacagacttagaaggtaacttttatggaccttttgttgacaggcaaacagcacaagcagctggtacggacacaactattacagttaatgttttagcttggttgtacgctgctgttataaatggagacaggtggtttctcaatcgatttaccacaactcttaatgactttaaccttgtggctatgaagtacaattatgaacctctaacacaagaccatgttgacatactaggacctctttctgctcaaactggaattgccgttttagatatgtgtgcttcattaaaagaattactgcaaaatggtatgaatggacgtaccatattgggtagtgctttattagaagatgaatttacaccttttgatgttgttagacaatgctcaggtgttactttccaaagtgcagtgaaaagaacaatcaagggtacacaccactggttgttactcacaattttgacttcacttttagttttagtccagagtactcaatggtctttgttcttttttttgtatgaaaatgcctttttaccttttgctatgggtattattgctatgtctgcttttgcaatgatgtttgtcaaacataagcatgcatttctctgtttgtttttgttaccttctcttgccactgtagcttattttaatatggtctatatgcctgctagttgggtgatgcgtattatgacatggttggatatggttgatactagtttgtctggttttaagctaaaagactgtgttatgtatgcatcagctgtagtgttactaatccttatgacagcaagaactgtgtatgatgatggtgctaggagagtgtggacacttatgaatgtcttgacactcgtttataaagtttattatggtaatgctttagatcaagccatttccatgtgggctcttataatctctgttacttctaactactcaggtgtagttacaactgtcatgtttttggccagaggtattgtttttatgtgtgttgagtattgccctattttcttcataactggtaatacacttcagtgtataatgctagtttattgtttcttaggctatttttgtacttgttactttggcctcttttgtttactcaaccgctactttagactgactcttggtgtttatgattacttagtttctacacaggagtttagatatatgaattcacagggactactcccacccaagaatagcatagatgccttcaaactcaacattaaattgttgggtgttggtggcaaaccttgtatcaaagtagccactgtacagtctaaaatgtcagatgtaaagtgcacatcagtagtcttactctcagttttgcaacaactcagagtagaatcatcatctaaattgtgggctcaatgtgtccagttacacaatgacattctcttagctaaagatactactgaagcctttgaaaaaatggtttcactactttctgttttgctttccatgcagggtgctgtagacataaacaagctttgtgaagaaatgctggacaacagggcaaccttacaagctatagcctcagagtttagttcccttccatcatatgcagcttttgctactgctcaagaagcttatgagcaggctgttgctaatggtgattctgaagttgttcttaaaaagttgaagaagtctttgaatgtggctaaatctgaatttgaccgtgatgcagccatgcaacgtaagttggaaaagatggctgatcaagctatgacccaaatgtataaacaggctagatctgaggacaagagggcaaaagttactagtgctatgcagacaatgcttttcactatgcttagaaagttggataatgatgcactcaacaacattatcaacaatgcaagagatggttgtgttcccttgaacataatacctcttacaacagcagccaaactaatggttgtcataccagactataacacatataaaaatacgtgtgatggtacaacatttacttatgcatcagcattgtgggaaatccaacaggttgtagatgcagatagtaaaattgttcaacttagtgaaattagtatggacaattcacctaatttagcatggcctcttattgtaacagctttaagggccaattctgctgtcaaattacagaataatgagcttagtcctgttgcactacgacagatgtcttgtgctgccggtactacacaaactgcttgcactgatgacaatgcgttagcttactacaacacaacaaagggaggtaggtttgtacttgcactgttatccgatttacaggatttgaaatgggctagattccctaagagtgatggaactggtactatctatacagaactggaaccaccttgtaggtttgttacagacacacctaaaggtcctaaagtgaagtatttatactttattaaaggattaaacaacctaaatagaggtatggtacttggtagtttagctgccacagtacgtctacaagctggtaatgcaacagaagtgcctgccaattcaactgtattatctttctgtgcttttgctgtagatgctgctaaagcttacaaagattatctagctagtgggggacaaccaatcactaattgtgttaagatgttgtgtacacacactggtactggtcaggcaataacagttacaccggaagccaatatggatcaagaatcctttggtggtgcatcgtgttgtctgtactgccgttgccacatagatcatccaaatcctaaaggattttgtgacttaaaaggtaagtatgtacaaatacctacaacttgtgctaatgaccctgtgggttttacacttaaaaacacagtctgtaccgtctgcggtatgtggaaaggttatggctgtagttgtgatcaactccgcgaacccatgcttcagtcagctgatgcacaatcgtttttaaacgggtttgcggtgtaagtgcagcccgtcttacaccgtgcggcacaggcactagtactgatgtcgtatacagggcttttgacatctacaatgataaagtagctggttttgctaaattcctaaaaactaattgttgtcgcttccaagaaaaggacgaagatgacaatttaattgattcttactttgtagttaagagacacactttctctaactaccaacatgaagaaacaatttataatttacttaaggattgtccagctgttgctaaacatgacttctttaagtttagaatagacggtgacatggtaccacatatatcacgtcaacgtcttactaaatacacaatggcagacctcgtctatgctttaaggcattttgatgaaggtaattgtgacacattaaaagaaatacttgtcacatacaattgttgtgatgatgattatttcaataaaaaggactggtatgattttgtagaaaacccagatatattacgcgtatacgccaacttaggtgaacgtgtacgccaagctttgttaaaaacagtacaattctgtgatgccatgcgaaatgctggtattgttggtgtactgacattagataatcaagatctcaatggtaactggtatgatttcggtgatttcatacaaaccacgccaggtagtggagttcctgttgtagattcttattattcattgttaatgcctatattaaccttgaccagggctttaactgcagagtcacatgttgacactgacttaacaaagccttacattaagtgggatttgttaaaatatgacttcacggaagagaggttaaaactctttgaccgttattttaaatattgggatcagacataccacccaaattgtgttaactgtttggatgacagatgcattctgcattgtgcaaactttaatgttttattctctacagtgttcccacctacaagttttggaccactagtgagaaaaatatttgttgatggtgttccatttgtagtttcaactggataccacttcagagagctaggtgttgtacataatcaggatgtaaacttacatagctctagacttagttttaaggaattacttgtgtatgctgctgaccctgctatgcacgctgcttctggtaatctattactagataaacgcactacgtgcttttcagtagctgcacttactaacaatgttgcttttcaaactgtcaaacccggtaattttaacaaagacttctatgactttgctgtgtctaagggtttctttaaggaaggaagttctgttgaattaaaacacttcttctttgctcaggatggtaatgctgctatcagcgattatgactactatcgttataatctaccaacaatgtgtgatatcagacaactactatttgtagttgaagttgttgataagtactttgattgttacgatggtggctgtattaatgctaaccaagtcatcgtcaacaacctagacaaatcagctggttttccatttaataaatggggtaaggctagactttattatgattcaatgagttatgaggatcaagatgcacttttcgcatatacaaaacgtaatgtcatccctactataactcaaatgaatcttaagtatgccattagtgcaaagaatagagctcgcaccgtagctggtgtctctatctgtagtactatgaccaatagacagtttcatcaaaaattattgaaatcaatagccgccactagaggagctactgtagtaattggaacaagcaaattctatggtggttggcacaacatgttaaaaactgtttatagtgatgtagaaaaccctcaccttatgggttgggattatcctaaatgtgatagagccatgcctaacatgcttagaattatggcctcacttgttcttgctcgcaaacatacaacgtgttgtagcttgtcacaccgtttctatagattagctaatgagtgtgctcaagtattgagtgaaatggtcatgtgtggcggttcactatatgttaaaccaggtggaacctcatcaggagatgccacaactgcttatgctaatagtgtttttaacatttgtcaagctgtcacggccaatgttaatgcacttttatctactgatggtaacaaaattgccgataagtatgtccgcaatttacaacacagactttatgagtgtctctatagaaatagagatgttgacacagactttgtgaatgagttttacgcatatttgcgtaaacatttctcaatgatgatactctctgacgatgctgttgtgtgtttcaatagcacttatgcatctcaaggtctagtggctagcataaagaactttaagtcagttctttattatcaaaacaatgtttttatgtctgaagcaaaatgttggactgagactgaccttactaaaggacctcatgaattttgctctcaacatacaatgctagttaaacagggtgatgattatgtgtaccttccttacccagatccatcaagaatcctaggggccggctgttttgtagatgatatcgtaaaaacagatggtacacttatgattgaacggttcgtgtctttagctatagatgcttacccacttactaaacatcctaatcaggagtatgctgatgtctttcatttgtacttacaatacataagaaagctacatgatgagttaacaggacacatgttagacatgtattctgttatgcttactaatgataacacttcaaggtattgggaacctgagttttatgaggctatgtacacaccgcatacagtcttacaggctgttggggcttgtgttctttgcaattcacagacttcattaagatgtggtgcttgcatacgtagaccattcttatgttgtaaatgctgttacgaccatgtcatatcaacatcacataaattagtcttgtctgttaatccgtatgtttgcaatgctccaggttgtgatgtcacagatgtgactcaactttacttaggaggtatgagctattattgtaaatcacataaaccacccattagttttccattgtgtgctaatggacaagtttttggtttatataaaaatacatgtgttggtagcgataatgttactgactttaatgcaattgcaacatgtgactggacaaatgctggtgattacattttagctaacacctgtactgaaagactcaagctttttgcagcagaaacgctcaaagctactgaggagacatttaaactgtcttatggtattgctactgtacgtgaagtgctgtctgacagagaattacatctttcatgggaagttggtaaacctagaccaccacttaaccgaaattatgtctttactggttatcgtgtaactaaaaacagtaaagtacaaataggagagtacacctttgaaaaaggtgactatggtgatgctgttgtttaccgaggtacaacaacttacaaattaaatgttggtgattattttgtgctgacatcacatacagtaatgccattaagtgcacctacactagtgccacaagagcactatgttagaattactggcttatacccaacactcaatatctcagatgagttttctagcaatgttgcaaattatcaaaaggttggtatgcaaaagtattctacactccagggaccacctggtactggtaagagtcattttgctattggcctagctctctactacccttctgctcgcatagtgtatacagcttgctctcatgccgctgttgatgcactatgtgagaaggcattaaaatatttgcctatagataaatgtagtagaattatacctgcacgtgctcgtgtagagtgttttgataaattcaaagtgaattcaacattagaacagtatgtcttttgtactgtaaatgcattgcctgagacgacagcagatatagttgtctttgatgaaatttcaatggccacaaattatgatttgagtgttgtcaatgccagattacgtgctaagcactatgtgtacattggcgaccctgctcaattacctgcaccacgcacattgctaactaagggcacactagaaccagaatatttcaattcagtgtgtagacttatgaaaactataggtccagacatgttcctcggaacttgtcggcgttgtcctgctgaaattgttgacactgtgagtgctttggtttatgataataagcttaaagcacataaagacaaatcagctcaatgctttaaaatgttttataagggtgttatcacgcatgatgtttcatctgcaattaacaggccacaaataggcgtggtaagagaattccttacacgtaaccctgcttggagaaaagctgtctttatttcaccttataattcacagaatgctgtagcctcaaagattttgggactaccaactcaaactgttgattcatcacagggctcagaatatgactatgtcatattcactcaaaccactgaaacagctcactcttgtaatgtaaacagatttaatgttgctattaccagagcaaaagtaggcatactttgcataatgtctgatagagacctttatgacaagttgcaatttacaagtcttgaaattccacgtaggaatgtggcaactttacaagctgaaaatgtaacaggactctttaaagattgtagtaaggtaatcactgggttacatcctacacaggcacctacacacctcagtgttgacactaaattcaaaactgaaggtttatgtgttgacatacctggcatacctaaggacatgacctatagaagactcatctctatgatgggttttaaaatgaattatcaagttaatggttaccctaacatgtttatcacccgcgaagaagctataagacatgtacgtgcatggattggcttcgatgtcgaggggtgtcatgctactagagaagctgttggtaccaatttacctttacagctaggtttttctacaggtgttaacctagttgctgtacctacaggttatgttgatacacctaataatacagatttttccagagttagtgctaaaccaccgcctggagatcaatttaaacacctcataccacttatgtacaaaggacttccttggaatgtagtgcgtataaagattgtacaaatgttaagtgacacacttaaaaatctctctgacagagtcgtatttgtcttatgggcacacggctttgagttgacatctatgaagtattttgtgaaaataggacctgagcgcacctgttgtctatgtgatagacgtgccacatgcttttccactgcttcagacacttatgcctgttggcatcattctattggatttgattacgtctataatccgtttatgattgatgttcaacaatggggttttacaggtaacctacaaagcaaccatgatctgtattgtcaagtccatggtaatgcacatgtagctagttgtgatgcaatcatgactaggtgtctagctgtccacgagtgctttgttaagcgtgttgactggactattgaatatcctataattggtgatgaactgaagattaatgcggcttgtagaaaggtacaacacatggttgttaaagctgcattattagcagacaaattcccagttcttcacgacattggtaaccctaaagctattaagtgtgtacctcaagctgatgtagaatggaagttctatgatgcacagccttgtagtgacaaagcttataaaatagaagaattattctattcttatgccacacattctgacaaattcacagctggtgtatgcctattttggaattgcaatgtcgatagatatcctgctaattccattgtttgtagatttgacactagagtgctatctaaccttaacttgcctggttgtgatggtggcagtttgtatgtaaataaacatgcattccacacaccagcttttgataaaagtgcttttgttaatttaaaacaattaccatttttctattactctgacagtccatgtgagtctcatggaaaacaagtagtgtcagatatagattatgtaccactaaagtctgctacgtgtataacacgttgcaatttaggtggtgctgtctgtagacatcatgctaatgagtacagattgtatctcgatgcttataacatgatgatctcagctggctttagcttgtgggtttacaaacaatttgatacttataacctctggaacacttttacaagacttcagagtttagaaaatgtggcttttaatgttgtaaataagggacactttgatggacaacagggtgaagtaccagtttctatcattaataacactgtttacacaaaagttgatggtgttgatgtagaattgtttgaaaataaaacaacattacctgttaatgtagcatttgagctttgggctaagcgcaacattaaaccagtaccagaggtgaaaatactcaataatttgggtgtggacattgctgctaatactgtgatctgggactacaaaagagatgctccagcacatatatctactattggtgtttgttctatgactgacatagccaagaaaccaactgaaacgatttgtgcaccactcactgtcttttttgatggtagagttgatggtcaagtagacttatttagaaatgcccgtaatggtgttcttattacagaaggtagtgttaaaggtttacaaccatctgtaggtcccaaacaagctagtcttaatggagtcacattaattggagaagccgtaaaaacacagttcaattattataagaaagttgatggtgttgtccaacaattacctgaaacttactttactcagagtagaaatttacaagaatttaaacccaggagtcaaatggaaattgatttcttagaattagctatggatgaattcattgaacggtataaattagaaggctatgccttcgaacatatcgtttatggagattttagtcatagtcagttaggtggtttacatctactgattggactagctaaacgttttaaggaatcaccttttgaattagaagattttattcctatggacagtacagttaaaaactatttcataacagatgcgcaaacaggttcatctaagtgtgtgtgttctgttattgatttattacttgatgattttgttgaaataataaaatcccaagatttatctgtagtttctaaggttgtcaaagtgactattgactatacagaaatttcatttatgctttggtgtaaagatggccatgtagaaacattttacccaaaattacaatctagtcaagcgtggcaaccgggtgttgctatgcctaatctttacaaaatgcaaagaatgctattagaaaagtgtgaccttcaaaattatggtgatagtgcaacattacctaaaggcataatgatgaatgtcgcaaaatatactcaactgtgtcaatatttaaacacattaacattagctgtaccctataatatgagagttatacattttggtgctggttctgataaaggagttgcaccaggtacagctgttttaagacagtggttgcctacgggtacgctgcttgtcgattcagatcttaatgactttgtctctgatgcagattcaactttgattggtgattgtgcaactgtacatacagctaataaatgggatctcattattagtgatatgtacgaccctaagactaaaaatgttacaaaagaaaatgactctaaagagggttttttcacttacatttgtgggtttatacaacaaaagctagctcttggaggttccgtggctataaagataacagaacattcttggaatgctgatctttataagctcatgggacacttcgcatggtggacagcctttgttactaatgtgaatgcgtcatcatctgaagcatttttaattggatgtaattatcttggcaaaccacgcgaacaaatagatggttatgtcatgcatgcaaattacatattttggaggaatacaaatccaattcagttgtcttcctattctttatttgacatgagtaaatttccccttaaattaaggggtactgctgttatgtctttaaaagaaggtcaaatcaatgatatgattttatctcttcttagtaaaggtagacttataattagagaaaacaacagagttgttatttctagtgatgttcttgttaacaactaaacgaacaatgtttgtttttcttgttttattgccactagtctctagtcagtgtgttaatcttacaaccagaactcaattaccccctgcatacactaattctttcacacgtggtgtttattaccctgacaaagttttcagatcctcagttttacattcaactcaggacttgttcttacctttcttttccaatgttacttggttccatgctatacatgtctctgggaccaatggtactaagaggtttgataaccctgtcctaccatttaatgatggtgtttattttgcttccactgagaagtctaacataataagaggctggatttttggtactactttagattcgaagacccagtccctacttattgttaataacgctactaatgttgttattaaagtctgtgaatttcaattttgtaatgatccatttttgggtgtttattaccacaaaaacaacaaaagttggatggaaagtgagttcagagtttattctagtgcgaataattgcacttttgaatatgtctctcagccttttcttatggaccttgaaggaaaacagggtaatttcaaaaatcttagggaatttgtgtttaagaatattgatggttattttaaaatatattctaagcacacgcctattaatttagtgcgtgatctccctcagggtttttcggctttagaaccattggtagatttgccaataggtattaacatcactaggtttcaaactttacttgctttacatagaagttatttgactcctggtgattcttcttcaggttggacagctggtgctgcagcttattatgtgggttatcttcaacctaggacttttctattaaaatataatgaaaatggaaccattacagatgctgtagactgtgcacttgaccctctctcagaaacaaagtgtacgttgaaatccttcactgtagaaaaaggaatctatcaaacttctaactttagagtccaaccaacagaatctattgttagatttcctaatattacaaacttgtgcccttttggtgaagtttttaacgccaccagatttgcatctgtttatgcttggaacaggaagagaatcagcaactgtgttgctgattattctgtcctatataattccgcatcattttccacttttaagtgttatggagtgtctcctactaaattaaatgatctctgctttactaatgtctatgcagattcatttgtaattagaggtgatgaagtcagacaaatcgctccagggcaaactggaaagattgctgattataattataaattaccagatgattttacaggctgcgttatagcttggaattctaacaatcttgattctaaggttggtggtaattataattacctgtatagattgtttaggaagtctaatctcaaaccttttgagagagatatttcaactgaaatctatcaggccggtagcacaccttgtaatggtgttgaaggttttaattgttactttcctttacaatcatatggtttccaacccactaatggtgttggttaccaaccatacagagtagtagtactttcttttgaacttctacatgcaccagcaactgtttgtggacctaaaaagtctactaatttggttaaaaacaaatgtgtcaatttcaacttcaatggtttaacaggcacaggtgttcttactgagtctaacaaaaagtttctgcctttccaacaatttggcagagacattgctgacactactgatgctgtccgtgatccacagacacttgagattcttgacattacaccatgttcttttggtggtgtcagtgttataacaccaggaacaaatacttctaaccaggttgctgttctttatcaggatgttaactgcacagaagtccctgttgctattcatgcagatcaacttactcctacttggcgtgtttattctacaggttctaatgtttttcaaacacgtgcaggctgtttaataggggctgaacatgtcaacaactcatatgagtgtgacatacccattggtgcaggtatatgcgctagttatcagactcagactaattctcctcggcgggcacgtagtgtagctagtcaatccatcattgcctacactatgtcacttggtgcagaaaattcagttgcttactctaataactctattgccatacccacaaattttactattagtgttaccacagaaattctaccagtgtctatgaccaagacatcagtagattgtacaatgtacatttgtggtgattcaactgaatgcagcaatcttttgttgcaatatggcagtttttgtacacaattaaaccgtgctttaactggaatagctgttgaacaagacaaaaacacccaagaagtttttgcacaagtcaaacaaatttacaaaacaccaccaattaaagattttggtggttttaatttttcacaaatattaccagatccatcaaaaccaagcaagaggtcatttattgaagatctacttttcaacaaagtgacacttgcagatgctggcttcatcaaacaatatggtgattgccttggtgatattgctgctagagacctcatttgtgcacaaaagtttaacggccttactgttttgccacctttgctcacagatgaaatgattgctcaatacacttctgcactgttagcgggtacaatcacttctggttggacctttggtgcaggtgctgcattacaaataccatttgctatgcaaatggcttataggtttaatggtattggagttacacagaatgttctctatgagaaccaaaaattgattgccaaccaatttaatagtgctattggcaaaattcaagactcactttcttccacagcaagtgcacttggaaaacttcaagatgtggtcaaccaaaatgcacaagctttaaacacgcttgttaaacaacttagctccaattttggtgcaatttcaagtgttttaaatgatatcctttcacgtcttgacaaagttgaggctgaagtgcaaattgataggttgatcacaggcagacttcaaagtttgcagacatatgtgactcaacaattaattagagctgcagaaatcagagcttctgctaatcttgctgctactaaaatgtcagagtgtgtacttggacaatcaaaaagagttgatttttgtggaaagggctatcatcttatgtccttccctcagtcagcacctcatggtgtagtcttcttgcatgtgacttatgtccctgcacaagaaaagaacttcacaactgctcctgccatttgtcatgatggaaaagcacactttcctcgtgaaggtgtctttgtttcaaatggcacacactggtttgtaacacaaaggaatttttatgaaccacaaatcattactacagacaacacatttgtgtctggtaactgtgatgttgtaataggaattgtcaacaacacagtttatgatcctttgcaacctgaattagactcattcaaggaggagttagataaatattttaagaatcatacatcaccagatgttgatttaggtgacatctctggcattaatgcttcagttgtaaacattcaaaaagaaattgaccgcctcaatgaggttgccaagaatttaaatgaatctctcatcgatctccaagaacttggaaagtatgagcagtatataaaatggccatggtacatttggctaggttttatagctggcttgattgccatagtaatggtgacaattatgctttgctgtatgaccagttgctgtagttgtctcaagggctgttgttcttgtggatcctgctgcaaatttgatgaagacgactctgagccagtgctcaaaggagtcaaattacattacacataaacgaacttatggatttgtttatgagaatcttcacaattggaactgtaactttgaagcaaggtgaaatcaaggatgctactccttcagattttgttcgcgctactgcaacgataccgatacaagcctcactccctttcggatggcttattgttggcgttgcacttcttgctgtttttcagagcgcttccaaaatcataaccctcaaaaagagatggcaactagcactctccaagggtgttcactttgtttgcaacttgctgttgttgtttgtaacagtttactcacaccttttgctcgttgctgctggccttgaagccccttttctctatctttatgctttagtctacttcttgcagagtataaactttgtaagaataataatgaggctttggctttgctggaaatgccgttccaaaaacccattactttatgatgccaactattttctttgctggcatactaattgttacgactattgtataccttacaatagtgtaacttcttcaattgtcattacttcaggtgatggcacaacaagtcctatttctgaacatgactaccagattggtggttatactgaaaaatgggaatctggagtaaaagactgtgttgtattacacagttacttcacttcagactattaccagctgtactcaactcaattgagtacagacactggtgttgaacatgttaccttcttcatctacaataaaattgttgatgagcctgaagaacatgtccaaattcacacaatcgacggttcatccggagttgttaatccagtaatggaaccaatttatgatgaaccgacgacgactactagcgtgcctttgtaagcacaagctgatgagtacgaacttatgtactcattcgtttcggaagagacaggtacgttaatagttaatagcgtacttctttttcttgctttcgtggtattcttgctagttacactagccatccttactgcgcttcgattgtgtgcgtactgctgcaatattgttaacgtgagtcttgtaaaaccttctttttacgtttactctcgtgttaaaaatctgaattcttctagagttcctgatcttctggtctaaacgaactaaatattatattagtttttctgtttggaactttaattttagccatggcagattccaacggtactattaccgttgaagagcttaaaaagctccttgaacaatggaacctagtaataggtttcctattccttacatggatttgtcttctacaatttgcctatgccaacaggaataggtttttgtatataattaagttaattttcctctggctgttatggccagtaactttagcttgttttgtgcttgctgctgtttacagaataaattggatcaccggtggaattgctatcgcaatggcttgtcttgtaggcttgatgtggctcagctacttcattgcttctttcagactgtttgcgcgtacgcgttccatgtggtcattcaatccagaaactaacattcttctcaacgtgccactccatggcactattctgaccagaccgcttctagaaagtgaactcgtaatcggagctgtgatccttcgtggacatcttcgtattgctggacaccatctaggacgctgtgacatcaaggacctgcctaaagaaatcactgttgctacatcacgaacgctttcttattacaaattgggagcttcgcagcgtgtagcaggtgactcaggttttgctgcatacagtcgctacaggattggcaactataaattaaacacagaccattccagtagcagtgacaatattgctttgcttgtacagtaagtgacaacagatgtttcatctcgttgactttcaggttactatagcagagatattactaattattatgaggacttttaaagtttccatttggaatcttgattacatcataaacctcataattaaaaatttatctaagtcactaactgagaataaatattctcaattagatgaagagcaaccaatggagattgattaaacgaacatgaaaattattcttttcttggcactgataacactcgctacttgtgagctttatcactaccaagagtgtgttagaggtacaacagtacttttaaaagaaccttgctcttctggaacatacgagggcaattcaccatttcatcctctagctgataacaaatttgcactgacttgctttagcactcaatttgcttttgcttgtcctgacggcgtaaaacacgtctatcagttacgtgccagatcagtttcacctaaactgttcatcagacaagaggaagttcaagaactttactctccaatttttcttattgttgcggcaatagtgtttataacactttgcttcacactcaaaagaaagacagaatgattgaactttcattaattgacttctatttgtgctttttagcctttctgctattccttgttttaattatgcttattatcttttggttctcacttgaactgcaagatcataatgaaacttgtcacgcctaaacgaacatgaaatttcttgttttcttaggaatcatcataactgtagctgcatttcaccaagaatgtagtttacagtcatgtactcaacatcaaccatatgtagttgatgacccgtgtcctattcacttctattctaaatggtatattagagtaggagctagaaaatcagcacctttaattgaattgtgcgtggatgaggctggttctaaatcacccattcagtacatcgatatcggtaattatacagtttcctgttcaccttttacaattaattgccaggaacctaaattgggtagtcttgtagtgcgttgttcgttctatgaagactttttagagtatcatgacgttcgtgttgttttagatttcatctaaacgaacaaactaaaatgtctgataatggaccccaaaatcagcgaaatgcaccccgcattacgtttggtggaccctcagattcaactggcagtaaccagaatggagaacgcagtggggcgcgatcaaaacaacgtcggccccaaggtttacccaataatactgcgtcttggttcaccgctctcactcaacatggcaaggaagaccttaaattccctcgaggacaaggcgttccaattaacaccaatagcagtccagatgaccaaattggctactaccgaagagctaccagacgaattcgtggtggtgacggtaaaatgaaagatctcagtccaagatggtatttctactacctaggaactgggccagaagctggacttccctatggtgctaacaaagacggcatcatatgggttgcaactgagggagccttgaatacaccaaaagatcacattggcacccgcaatcctgctaacaatgctgcaatcgtgctacaacttcctcaaggaacaacattgccaaaaggcttctacgcagaagggagcagaggcggcagtcaagcctcttctcgttcctcatcacgtagtcgcaacagttcaagaaattcaactccaggcagcagtaggggaacttctcctgctagaatggctggcaatggcggtgatgctgctcttgctttgctgctgcttgacagattgaaccagcttgagagcaaaatgtctggtaaaggccaacaacaacaaggccaaactgtcactaagaaatctgctgctgaggcttctaagaagcctcggcaaaaacgtactgccactaaagcatacaatgtaacacaagcttttggcagacgtggtccagaacaaacccaaggaaattttggggaccaggaactaatcagacaaggaactgattacaaacattggccgcaaattgcacaatttgcccccagcgcttcagcgttcttcggaatgtcgcgcattggcatggaagtcacaccttcgggaacgtggttgacctacacaggtgccatcaaattggatgacaaagatccaaatttcaaagatcaagtcattttgctgaataagcatattgacgcatacaaaacattcccaccaacagagcctaaaaaggacaaaaagaagaaggctgatgaaactcaagccttaccgcagagacagaagaaacagcaaactgtgactcttcttcctgctgcagatttggatgatttctccaaacaattgcaacaatccatgagcagtgctgactcaactcaggcctaaactcatgcagaccacacaaggcagatgggctatataaacgttttcgcttttccgtttacgatatatagtctactcttgtgcagaatgaattctcgtaactacatagcacaagtagatgtagttaactttaatctcacatagcaatctttaatcagtgtgtaacattagggaggacttgaaagagccaccacattttcaccgaggccacgcggagtacgatcgagtgtacagtgaacaatgctagggagagctgcctatatggaagagccctaatgtgtaaaattaattttagtagtgctatccccatgtgattttaatagcttcttaggagaatgacaaaaaaaaaaaa

SEQ ID NO: 2 - RNA, 1038 nt, Artificial Sequence
  Synthetic oligonucleotide
gggcgaauuggguaccgggcccccccucgaggucgacgguaucgauaagcuugauaucgaauuccugcagcccgggggauccagcuuggcacugauccuuaugaagauuuucaagaaaacuggaacacuaaacauagcagugguguuacccgugaacucaugcgugagcuuaacggaggggcauacacucgcuaugucgauaacaacuucuguggcccugauggcuacccucuugagugcauuaaagaccuucuagcacgugcugguaaagcuucaugcacuuuguccgaacaacuggacuuuauugacacuaagagggguguauacugcugccgugaacaugagcaugaaauugcuugguacacggaacguucugaaaagagcuaugaauugcagacaccuuuugaaauuaaauuggcaaagaaauuugacaccuucaauggggaauguccaaauuuuguauuucccuuaaauuccauaaucaagacuauucaaccaaggguugaaaagaaaaagcuugauggcuuuauggguagaauucgaucugucuauccaguugcgucaccaaaugaaugcaaccaaaugugccuuucaacucucaugaagugugaucauuguggugaaacuucauggcagacgggcgauuuuguuaaagccacuugcgaauuuuguggcacugagaauuugacuaaagaaggugccacuacuugugguuacuuaccccaaaaugcuguuguuaaaauuuauuguccagcaugucacaauucagaaguaggaccugagcauagucuugccgaauaccauaaugaaucuggcuugaaaaccauucuucguaaggguggucgcacuauugccuuuggaggcuguguguucucuuauguugguugccauaacaagugugccuauuggguuccacgugcuagcgcuaacauagguuguaaccauacagguguuguuggagaagguuccgaaggucuuaaugacaaccuucuugaaauacuccaaaaagagaaagucaacaucaauauuguugcggcc

SEQ ID NO: 3 - RNA, 1162 nt, Artificial Sequence
  Synthetic oligonucleotide
gggcgaauuggguaccgggcccccccucgaggucgacgguaucgauaagcuugauaucgaauuccugcagcccgggggaucccaguaaaacaacuguagcgucacuuaucaacacacuuaacgaucuaaaugaaacucuuguuacaaugccacuuggcuauguaacacauggcuuaaauuuggaagaagcugcucgguauaugagaucucucaaagugccagcuacaguuucuguuucuucaccugaugcuguuacagcguauaaugguuaucuuacuucuucuucuaaaacaccugaagaacauuuuauugaaaccaucucacuugcugguuccuauaaagauugguccuauucuggacaaucuacacaacuagguauagaauuucuuaagagaggugauaaaaguguauauuacacuaguaauccuaccacauuccaccuagauggugaaguuaucaccuuugacaaucuuaagacacuucuuucuuugagagaagugaggacuauuaagguguuuacaacaguagacaacauuaaccuccacacgcaaguuguggacaugucaaugacauauggacaacaguuugguccaacuuauuuggauggagcugauguuacuaaaauaaaaccucauaauucacaugaagguaaaacauuuuauguuuuaccuaaugaugacacucuacguguugaggcuuuugaguacuaccacacaacugauccuaguuuucuggguagguacaugucagcauuaaaucacacuaaaaaguggaaauacccacaaguuaaugguuuaacuucuauuaaaugggcagauaacaacuguuaucuugccacugcauuguuaacacuccaacaaauagaguugaaguuuaauccaccugcucuacaagaugcuuauuacagagcaagggcuggugaagcugcuaacuuuugugcacuuaucuuagccuacuguaauaagacaguaggugaguuaggugauguuagagaaacaaugaguuacuuguuucaacaugccaauuuagauucuugcaaaagagucuugaacgugguguguaaaacuuguggacaacagcagacaacccuuaaggguguagaagcuguuauguacaugggcacacuuucuuaugaacaauuuaagaaagguguucagcggcc

SEQ ID NO: 4 - DNA, 20 bp, Artificial Sequence
  Synthetic oligonucleotide
aggtcggtactaacatcaag

SEQ ID NO: 5 - DNA, 19 bp, Artificial Sequence
  Synthetic oligonucleotide
cacgttgtctggaagtttg

SEQ ID NO: 6 - DNA, 23 bp, Artificial Sequence
  Synthetic oligonucleotide
tagatggccgtctgtcgtatcca

SEQ ID NO: 7 - DNA, 49 bp, Artificial Sequence
  Synthetic oligonucleotide
  promoter (1)..(27)
aatttaatacgactcactatagggagagatgattgacttgtgattccgc

SEQ ID NO: 8 - DNA, 19 bp, Artificial Sequence
  Synthetic oligonucleotide
gattatataggacgacaag

SEQ ID NO: 9 - DNA, 18 bp, Artificial Sequence
  Synthetic oligonucleotide
ggugcgaauugggacaug

SEQ ID NO: 10 - DNA, 57 bp, Artificial Sequence
  Synthetic oligonucleotide
  misc_feature (25)..(57): Capture Probe Tail
cguucacuauuggucucugcauuctttaaaaaaaaaaaaaaaaaaaaaaaaaaaaaa

SEQ ID NO: 11 - DNA, 27 bp, Artificial Sequence
  Synthetic oligonucleotide
  promoter (1)..(27)
aatttaatacgactcactatagggaga

SEQ ID NO: 12 - DNA, 21 bp, Artificial Sequence
  Synthetic oligonucleotide
cttgatggctttatgggtaga

SEQ ID NO: 13 - DNA, 23 bp, Artificial Sequence
  Synthetic oligonucleotide
gagttgaaaggcacatttggttg

SEQ ID NO: 14 - DNA, 26 bp, Artificial Sequence
  Synthetic oligonucleotide
atctgtctatccagttgcgtcaccaa

SEQ ID NO: 15 - DNA, 21 bp, Artificial Sequence
  Synthetic oligonucleotide
gaagctgctcggtatatgaga

SEQ ID NO: 16 - DNA, 24 bp, Artificial Sequence
  Synthetic oligonucleotide
gaagtaagataaccattatacgct

SEQ ID NO: 17 - DNA, 27 bp, Artificial Sequence
  Synthetic oligonucleotide
tgccagctacagtttctgtttcttcac

SEQ ID NO: 18 - DNA, 27 bp, Artificial Sequence
  Synthetic oligonucleotide
cttgatggctttatgggtagaattcga

SEQ ID NO: 19 - DNA, 21 bp, Artificial Sequence
  Synthetic oligonucleotide
gcttgatggctttatgggtag

SEQ ID NO: 20 - DNA, 18 bp, Artificial Sequence
  Synthetic oligonucleotide
gctttatgggtagaattc

SEQ ID NO: 21 - DNA, 25 bp, Artificial Sequence
  Synthetic oligonucleotide
gcttgatggctttatgggtagaatt

SEQ ID NO: 22 - DNA, 23 bp, Artificial Sequence
  Synthetic oligonucleotide
ggaagaagctgctcggtatatga

SEQ ID NO: 23 - DNA, 23 bp, Artificial Sequence
  Synthetic oligonucleotide
ctgctcggtatatgagatctctc

SEQ ID NO: 24 - DNA, 20 bp, Artificial Sequence
  Synthetic oligonucleotide
ctcggtatatgagatctctc

SEQ ID NO: 25 - DNA, 22 bp, Artificial Sequence
  Synthetic oligonucleotide
gtatatgagatctctcaaagtg

SEQ ID NO: 26 - DNA, 28 bp, Artificial Sequence
  Synthetic oligonucleotide
gcttgatggctttatgggtagaattcga

SEQ ID NO: 27 - DNA, 20 bp, Artificial Sequence
  Synthetic oligonucleotide
cttgatggctttatgggtag

SEQ ID NO: 28 - DNA, 13 bp, Artificial Sequence
  Synthetic oligonucleotide
gctttatgggtag

SEQ ID NO: 29 - DNA, 37 bp, Artificial Sequence
  Synthetic oligonucleotide
ggaagaagctgctcggtatatgagatctctcaaagtg

SEQ ID NO: 30 - DNA, 15 bp, Artificial Sequence
  Synthetic oligonucleotide
ctgctcggtatatga

SEQ ID NO: 31 - DNA, 14 bp, Artificial Sequence
  Synthetic oligonucleotide
ctcggtatatgaga

SEQ ID NO: 32 - DNA, 26 bp, Artificial Sequence
  Synthetic oligonucleotide
aucugucuauccaguugcgucaccaa

SEQ ID NO: 33 - DNA, 24 bp, Artificial Sequence
  Synthetic oligonucleotide
aucugucuauccaguugcgucacc

SEQ ID NO: 34 - DNA, 23 bp, Artificial Sequence
  Synthetic oligonucleotide
aucugucuauccaguugcgucac

SEQ ID NO: 35 - DNA, 24 bp, Artificial Sequence
  Synthetic oligonucleotide
ucugucuauccaguugcgucacca

SEQ ID NO: 36 - DNA, 23 bp, Artificial Sequence
  Synthetic oligonucleotide
ucugucuauccaguugcgucacc

SEQ ID NO: 37 - DNA, 22 bp, Artificial Sequence
  Synthetic oligonucleotide
ucugucuauccaguugcgucac

SEQ ID NO: 38 - DNA, 20 bp, Artificial Sequence
  Synthetic oligonucleotide
cuauccaguugcgucaccaa

SEQ ID NO: 39 - DNA, 19 bp, Artificial Sequence
  Synthetic oligonucleotide
cuauccaguugcgucacca

SEQ ID NO: 40 - DNA, 22 bp, Artificial Sequence
  Synthetic oligonucleotide
gucuauccaguugcgucaccaa

SEQ ID NO: 41 - DNA, 24 bp, Artificial Sequence
  Synthetic oligonucleotide
ucgaucugucuauccaguugcguc

SEQ ID NO: 42 - DNA, 34 bp, Artificial Sequence
  Synthetic oligonucleotide
auuuggugacgcaacuggauagacagaucgaauu

SEQ ID NO: 43 - DNA, 27 bp, Artificial Sequence
  Synthetic oligonucleotide
gccagcuacaguuucuguuucuucacc

SEQ ID NO: 44 - DNA, 29 bp, Artificial Sequence
  Synthetic oligonucleotide
gugccagcuacaguuucuguuucuucacc

SEQ ID NO: 45 - DNA, 28 bp, Artificial Sequence
  Synthetic oligonucleotide
gugccagcuacaguuucuguuucuucac

SEQ ID NO: 46 - DNA, 27 bp, Artificial Sequence
  Synthetic oligonucleotide
caaagugccagcuacaguuucuguuuc

SEQ ID NO: 47 - DNA, 26 bp, Artificial Sequence
  Synthetic oligonucleotide
caaagugccagcuacaguuucuguuu

SEQ ID NO: 48 - DNA, 27 bp, Artificial Sequence
  Synthetic oligonucleotide
gugccagcuacaguuucuguuucuuca

SEQ ID NO: 49 - DNA, 39 bp, Artificial Sequence
  Synthetic oligonucleotide
ucaggugaagaaacagaaacuguagcuggcacuuugaga

SEQ ID NO: 50 - DNA, 40 bp, Artificial Sequence
  Synthetic oligonucleotide
aattcgatctgtctatccagttgcgtcaccaaatgaatgc

SEQ ID NO: 51 - DNA, 21 bp, Artificial Sequence
  Synthetic oligonucleotide
atctgtctatccagttgcgtc

SEQ ID NO: 52 - DNA, 17 bp, Artificial Sequence
  Synthetic oligonucleotide
gtctatccagttgcgtc

SEQ ID NO: 53 - DNA, 22 bp, Artificial Sequence
  Synthetic oligonucleotide
gtctatccagttgcgtcaccaa

SEQ ID NO: 54 - DNA, 43 bp, Artificial Sequence
  Synthetic oligonucleotide
tctcaaagtgccagctacagtttctgtttcttcacctgatgct

SEQ ID NO: 55 - DNA, 20 bp, Artificial Sequence
  Synthetic oligonucleotide
gccagcuacaguuucuguuu

SEQ ID NO: 56 - DNA, 27 bp, Artificial Sequence
  Synthetic oligonucleotide
gtgccagctacagtttctgtttcttca

SEQ ID NO: 57 - DNA, 50 bp, Artificial Sequence
  Synthetic oligonucleotide
  promoter (1)..(27)
aatttaatacgactcactatagggagagagttgaaaggcacatttggttg

SEQ ID NO: 58 - DNA, 48 bp, Artificial Sequence
  Synthetic oligonucleotide
  promoter (1)..(27)
aatttaatacgactcactatagggagagagagttgaaaggcacatttg

SEQ ID NO: 59 - DNA, 45 bp, Artificial Sequence
  Synthetic oligonucleotide
  promoter (1)..(27)
aatttaatacgactcactatagggagaatgagagttgaaaggcac

SEQ ID NO: 60 - DNA, 51 bp, Artificial Sequence
  Synthetic oligonucleotide
  promoter (1)..(27)
aatttaatacgactcactatagggagacacacttcatgagagttgaaaggc

SEQ ID NO: 61 - DNA, 47 bp, Artificial Sequence
  Synthetic oligonucleotide
  promoter (1)..(27)
aatttaatacgactcactatagggagacttcatgagagttgaaaggc

SEQ ID NO: 62 - DNA, 49 bp, Artificial Sequence
  Synthetic oligonucleotide
  promoter (1)..(27)
aatttaatacgactcactatagggagacacacttcatgagagttgaaag

SEQ ID NO: 63 - DNA, 50 bp, Artificial Sequence
  Synthetic oligonucleotide
  promoter (1)..(27)
aatttaatacgactcactatagggagaccattatacgctgtaacagcatc

SEQ ID NO: 64 - DNA, 47 bp, Artificial Sequence
  Synthetic oligonucleotide
  promoter (1)..(27)
aatttaatacgactcactatagggagaccattatacgctgtaacagc

SEQ ID NO: 65 - DNA, 45 bp, Artificial Sequence
  Synthetic oligonucleotide
  promoter (1)..(27)
aatttaatacgactcactatagggagagataaccattatacgctg

SEQ ID NO: 66 - DNA, 43 bp, Artificial Sequence
  Synthetic oligonucleotide
  promoter (1)..(27)
aatttaatacgactcactatagggagagaagaagtaagataac

SEQ ID NO: 67 - DNA, 53 bp, Artificial Sequence
  Synthetic oligonucleotide
  promoter (1)..(27)
aatttaatacgactcactatagggagaagaagaagtaagataaccattatacg

SEQ ID NO: 68 - DNA, 54 bp, Artificial Sequence
  Synthetic oligonucleotide
  promoter (1)..(27)
aatttaatacgactcactataggggaagaagaagtaagataaccattatacgct

SEQ ID NO: 69 - DNA, 51 bp, Artificial Sequence
  Synthetic oligonucleotide
  promoter (1)..(27)
aatttaatacgactcactatagggagagaagaagtaagataaccattatac

SEQ ID NO: 70 - DNA, 47 bp, Artificial Sequence
  Synthetic oligonucleotide
  promoter (1)..(27)
aatttaatacgactcactatagggagagtaagataaccattatacgc

SEQ ID NO: 71 - DNA, 21 bp, Artificial Sequence
  Synthetic oligonucleotide
gagagttgaaaggcacatttg

SEQ ID NO: 72 - DNA, 18 bp, Artificial Sequence
  Synthetic oligonucleotide
atgagagttgaaaggcac

SEQ ID NO: 73 - DNA, 24 bp, Artificial Sequence
  Synthetic oligonucleotide
cacacttcatgagagttgaaaggc

SEQ ID NO: 74 - DNA, 20 bp, Artificial Sequence
  Synthetic oligonucleotide
cttcatgagagttgaaaggc

SEQ ID NO: 75 - DNA, 22 bp, Artificial Sequence
  Synthetic oligonucleotide
cacacttcatgagagttgaaag

SEQ ID NO: 76 - DNA, 23 bp, Artificial Sequence
  Synthetic oligonucleotide
ccattatacgctgtaacagcatc

SEQ ID NO: 77 - DNA, 20 bp, Artificial Sequence
  Synthetic oligonucleotide
ccattatacgctgtaacagc

SEQ ID NO: 78 - DNA, 51 bp, Artificial Sequence
  Synthetic oligonucleotide
  promoter (1)..(27)
aatttaatacgactcactatagggagagaagtaagataaccattatacgct

SEQ ID NO: 79 - DNA, 18 bp, Artificial Sequence
  Synthetic oligonucleotide
gataaccattatacgctg

SEQ ID NO: 80 - DNA, 16 bp, Artificial Sequence
  Synthetic oligonucleotide
gaagaagtaagataac

SEQ ID NO: 81 - DNA, 26 bp, Artificial Sequence
  Synthetic oligonucleotide
agaagaagtaagataaccattatacg

SEQ ID NO: 82 - DNA, 27 bp, Artificial Sequence
  Synthetic oligonucleotide
gaagaagtaagataaccattatacgct

SEQ ID NO: 83 - DNA, 24 bp, Artificial Sequence
  Synthetic oligonucleotide
gaagaagtaagataaccattatac

SEQ ID NO: 84 - DNA, 20 bp, Artificial Sequence
  Synthetic oligonucleotide
gtaagataaccattatacgc

SEQ ID NO: 85 - DNA, 35 bp, Artificial Sequence
  Synthetic oligonucleotide
cacacttcatgagagttgaaaggcacatttggttg

SEQ ID NO: 86 - DNA, 10 bp, Artificial Sequence
  Synthetic oligonucleotide
gagttgaaag

SEQ ID NO: 87 - DNA, 12 bp, Artificial Sequence
  Synthetic oligonucleotide
gagttgaaaggc

SEQ ID NO: 88 - DNA, 19 bp, Artificial Sequence
  Synthetic oligonucleotide
gagttgaaaggcacatttg

SEQ ID NO: 89 - DNA, 39 bp, Artificial Sequence
  Synthetic oligonucleotide
agaagaagtaagataaccattatacgctgtaacagcatc

SEQ ID NO: 90 - DNA, 15 bp, Artificial Sequence
  Synthetic oligonucleotide
gataaccattatacg

SEQ ID NO: 91 - DNA, 55 bp, Artificial Sequence
  Synthetic oligonucleotide
  misc_feature (23)..(55): Capture Probe Tail
gucuugauuauggaauuuaaggtttaaaaaaaaaaaaaaaaaaaaaaaaaaaaaa

SEQ ID NO: 92 - DNA, 57 bp, Artificial Sequence
  Synthetic oligonucleotide
  misc_feature (25)..(57): Capture Probe Tail
caaguaguggcaccuucuuuaguctttaaaaaaaaaaaaaaaaaaaaaaaaaaaaaa

SEQ ID NO: 93 - DNA, 54 bp, Artificial Sequence
  Synthetic oligonucleotide
  misc_feature (25)..(54): Capture Probe Tail
cugaauugugacaugcuggacuuuaaaaaaaaaaaaaaaaaaaaaaaaaaaaaa

SEQ ID NO: 94 - DNA, 57 bp, Artificial Sequence
  Synthetic oligonucleotide
  misc_feature (25)..(57): Capture Probe Tail
gccagauucauuaugguauucggctttaaaaaaaaaaaaaaaaaaaaaaaaaaaaaa

SEQ ID NO: 95 - DNA, 55 bp, Artificial Sequence
  Synthetic oligonucleotide
  misc_feature (23)..(55): Capture Probe Tail
ccuaguuguguagauuguccagtttaaaaaaaaaaaaaaaaaaaaaaaaaaaaaa

SEQ ID NO: 96 - DNA, 55 bp, Artificial Sequence
  Synthetic oligonucleotide
  misc_feature (23)..(55): Capture Probe Tail
gguggaaugugguaggauuacutttaaaaaaaaaaaaaaaaaaaaaaaaaaaaaa

SEQ ID NO: 97 - DNA, 22 bp, Artificial Sequence
  Synthetic oligonucleotide
gucuugauuauggaauuuaagg

SEQ ID NO: 98 - DNA, 24 bp, Artificial Sequence
  Synthetic oligonucleotide
caaguaguggcaccuucuuuaguc

SEQ ID NO: 99 - DNA, 21 bp, Artificial Sequence
  Synthetic oligonucleotide
cugaauugugacaugcuggac

SEQ ID NO: 100 - DNA, 24 bp, Artificial Sequence
  Synthetic oligonucleotide
gccagauucauuaugguauucggc

SEQ ID NO: 101 - DNA, 22 bp, Artificial Sequence
  Synthetic oligonucleotide
ccuaguuguguagauuguccag

SEQ ID NO: 102 - DNA, 22 bp, Artificial Sequence
  Synthetic oligonucleotide
gguggaaugugguaggauuacu

SEQ ID NO: 103 - DNA, 26 bp, Artificial Sequence
  Synthetic oligonucleotide
ggucuauccaguugcgucaccagacc

SEQ ID NO: 104 - DNA, 32 bp, Artificial Sequence
  Synthetic oligonucleotide
cugucuauccaguugcgucaccaaauggacag

SEQ ID NO: 105 - DNA, 30 bp, Artificial Sequence
  Synthetic oligonucleotide
ccagcuacaguuucuguuucuucacgcugg

SEQ ID NO: 106 - DNA, 30 bp, Artificial Sequence
  Synthetic oligonucleotide
gcuacaguuucuguuucuucaccugguagc

SEQ ID NO: 107 - DNA, 21 bp, Artificial Sequence
  Synthetic oligonucleotide
ggucuauccaguugcgucacc

SEQ ID NO: 108 - DNA, 27 bp, Artificial Sequence
  Synthetic oligonucleotide
cugucuauccaguugcgucaccaaaug

SEQ ID NO: 109 - DNA, 25 bp, Artificial Sequence
  Synthetic oligonucleotide
ccagcuacaguuucuguuucuucac

SEQ ID NO: 110 - DNA, 25 bp, Artificial Sequence
  Synthetic oligonucleotide
gcuacaguuucuguuucuucaccug

SEQ ID NO: 111 - DNA, 16 bp, Artificial Sequence
  Synthetic oligonucleotide
gtatatgagatctctc

SEQ ID NO: 112 - DNA, 15 bp, Artificial Sequence
  Synthetic oligonucleotide
ccattatacgctgta

SEQ ID NO: 113 - DNA, 10 bp, Artificial Sequence
  Synthetic oligonucleotide
gtaagataac

SEQ ID NO: 114 - DNA, 16 bp, Artificial Sequence
  Synthetic oligonucleotide
ctatccagttgcgtca

SEQ ID NO: 115 - DNA, 16 bp, Artificial Sequence
  Synthetic oligonucleotide
gctacagtttctgttt